European Patent Specification EP 4 041 727 B1, published May 20, 2026. Title: ATF6 MODULATORS AND USES THEREOF. Applicant: Black Belt Tx Ltd. The sequence listing filed with the application follows.

SEQUENCE LISTING (1 sequence)

SEQ ID NO: 1 - DNA, 19 bp, Artificial Sequence
  Synthetic Construct
ccaatcggcggcggccacg